European Patent Specification EP 3 772 929 B1, published November 15, 2023. Title: NON-HUMAN ANIMALS COMPRISING A HUMANIZED COAGULATION FACTOR 12 LOCUS. Applicant: Regeneron Pharmaceuticals, Inc. The sequence listing filed with the application follows.

SEQUENCE LISTING (84 sequences)

SEQ ID NO: 1 - protein, 597 aa, Mus musculus
  MISC_FEATURE (1)..(19): Signal Peptide
  MISC_FEATURE (20)..(354): Heavy Chain
  MISC_FEATURE (355)..(597): Light Chain
MTALLFLGSLLMSLDLTLSAPPWKDSKKFKDAPDGPTVVLTVDGRLCHFPFQYHRQLHHKCIHKRRPGSRPWCATTPNFDEDQQWGYCLEPKKVKDHCSKHNPCHKGGTCINTPNGPHCLCPEHLTGKHCQKEKCFEPQLLKFFHENELWFRTGPGGVARCECKGSEAHCKPVASQACSINPCLNGGSCLLVEDHPLCRCPTGYTGYFCDLDLWATCYEGRGLSYRGQAGTTQSGAPCQRWTVEATYRNMTEKQALSWGLGHHAFCRNPDNDTRPWCFVWSGDRLSWDYCGLEQCQTPTFAPLVVPESQEESPSQAPSLSHAPNDSTDHQTSLSKTNTMGCGQRFRKGLSSFMRVVGGLVALPGSHPYIAALYWGNNFCAGSLIAPCWVLTAAHCLQNRPAPEELTVVLGQDRHNQSCEWCQTLAVRSYRLHEGFSSITYQHDLALLRLQESKTNSCAILSPHVQPVCLPSGAAPPSETVLCEVAGWGHQFEGAEEYSTFLQEAQVPFIALDRCSNSNVHGDAILPGMLCAGFLEGGTDACQGDSGGPLVCEEGTAEHQLTLRGVISWGSGCGDRNKPGVYTDVANYLAWIQKHIAS

SEQ ID NO: 2 - protein, 19 aa, Mus musculus
MTALLFLGSLLMSLDLTLS

SEQ ID NO: 3 - protein, 335 aa, Mus musculus
APPWKDSKKFKDAPDGPTVVLTVDGRLCHFPFQYHRQLHHKCIHKRRPGSRPWCATTPNFDEDQQWGYCLEPKKVKDHCSKHNPCHKGGTCINTPNGPHCLCPEHLTGKHCQKEKCFEPQLLKFFHENELWFRTGPGGVARCECKGSEAHCKPVASQACSINPCLNGGSCLLVEDHPLCRCPTGYTGYFCDLDLWATCYEGRGLSYRGQAGTTQSGAPCQRWTVEATYRNMTEKQALSWGLGHHAFCRNPDNDTRPWCFVWSGDRLSWDYCGLEQCQTPTFAPLVVPESQEESPSQAPSLSHAPNDSTDHQTSLSKTNTMGCGQRFRKGLSSFMR

SEQ ID NO: 4 - protein, 243 aa, Mus musculus
VVGGLVALPGSHPYIAALYWGNNFCAGSLIAPCWVLTAAHCLQNRPAPEELTVVLGQDRHNQSCEWCQTLAVRSYRLHEGFSSITYQHDLALLRLQESKTNSCAILSPHVQPVCLPSGAAPPSETVLCEVAGWGHQFEGAEEYSTFLQEAQVPFIALDRCSNSNVHGDAILPGMLCAGFLEGGTDACQGDSGGPLVCEEGTAEHQLTLRGVISWGSGCGDRNKPGVYTDVANYLAWIQKHIAS

SEQ ID NO: 5 - protein, 615 aa, Homo sapiens
  MISC_FEATURE (1)..(19): Signal Peptide
  MISC_FEATURE (20)..(372): Heavy Chain
  MISC_FEATURE (373)..(615): Light Chain
MRALLLLGFLLVSLESTLSIPPWEAPKEHKYKAEEHTVVLTVTGEPCHFPFQYHRQLYHKCTHKGRPGPQPWCATTPNFDQDQRWGYCLEPKKVKDHCSKHSPCQKGGTCVNMPSGPHCLCPQHLTGNHCQKEKCFEPQLLRFFHKNEIWYRTEQAAVARCQCKGPDAHCQRLASQACRTNPCLHGGRCLEVEGHRLCHCPVGYTGPFCDVDTKASCYDGRGLSYRGLARTTLSGAPCQPWASEATYRNVTAEQARNWGLGGHAFCRNPDNDIRPWCFVLNRDRLSWEYCDLAQCQTPTQAAPPTPVSPRLHVPLMPAQPAPPKPQPTTRTPPQSQTPGALPAKREQPPSLTRNGPLSCGQRLRKSLSSMTRVVGGLVALRGAHPYIAALYWGHSFCAGSLIAPCWVLTAAHCLQDRPAPEDLTVVLGQERRNHSCEPCQTLAVRSYRLHEAFSPVSYQHDLALLRLQEDADGSCALLSPYVQPVCLPSGAARPSETTLCQVAGWGHQFEGAEEYASFLQEAQVPFLSLERCSAPDVHGSSILPGMLCAGFLEGGTDACQGDSGGPLVCEDQAAERRLTLQGIISWGSGCGDRNKPGVYTDVAYYLAWIREHTVS

SEQ ID NO: 6 - protein, 19 aa, Homo sapiens
MRALLLLGFLLVSLESTLS

SEQ ID NO: 7 - protein, 353 aa, Homo sapiens
IPPWEAPKEHKYKAEEHTVVLTVTGEPCHFPFQYHRQLYHKCTHKGRPGPQPWCATTPNFDQDQRWGYCLEPKKVKDHCSKHSPCQKGGTCVNMPSGPHCLCPQHLTGNHCQKEKCFEPQLLRFFHKNEIWYRTEQAAVARCQCKGPDAHCQRLASQACRTNPCLHGGRCLEVEGHRLCHCPVGYTGPFCDVDTKASCYDGRGLSYRGLARTTLSGAPCQPWASEATYRNVTAEQARNWGLGGHAFCRNPDNDIRPWCFVLNRDRLSWEYCDLAQCQTPTQAAPPTPVSPRLHVPLMPAQPAPPKPQPTTRTPPQSQTPGALPAKREQPPSLTRNGPLSCGQRLRKSLSSMTR

SEQ ID NO: 8 - protein, 243 aa, Homo sapiens
VVGGLVALRGAHPYIAALYWGHSFCAGSLIAPCWVLTAAHCLQDRPAPEDLTVVLGQERRNHSCEPCQTLAVRSYRLHEAFSPVSYQHDLALLRLQEDADGSCALLSPYVQPVCLPSGAARPSETTLCQVAGWGHQFEGAEEYASFLQEAQVPFLSLERCSAPDVHGSSILPGMLCAGFLEGGTDACQGDSGGPLVCEDQAAERRLTLQGIISWGSGCGDRNKPGVYTDVAYYLAWIREHTVS

SEQ ID NO: 9 - DNA, 1794 bp, Mus musculus
  misc_feature (1)..(57): Signal Peptide
  misc_feature (58)..(1062): Heavy Chain
  misc_feature (1063)..(1791): Light Chain
atgacggctctgttgttcctggggtctctgctgatgagtctggatctgacactttcggctccaccatggaaagactccaagaaatttaaggacgcacctgatgggcccacagtggttctcactgtggatgggaggctctgccattttccctttcagtaccaccgtcagctacaccacaaatgcatccacaaaaggcggccaggctcccgcccctggtgtgctaccacccccaactttgatgaagatcagcaatggggatactgcttggagcccaagaaagtgaaagaccattgcagcaaacacaacccgtgccacaaaggagggacatgtatcaacacccccaatgggccacactgtctctgccctgaacacctcactgggaaacattgccagaaagagaaatgctttgagcctcagcttctcaagttcttccacgagaatgagctatggtttagaacggggccaggaggtgtggccaggtgcgagtgcaaaggttctgaggctcactgcaagccggtggccagccaggcctgcagcatcaatccgtgccttaatgggggcagctgcctcctcgtggaggaccacccactgtgccgttgccctacaggctacactggatatttttgcgacttggacctttgggcgacctgctatgaaggcagggggctcagctaccggggccaggctggaactacgcaatcgggtgcgccatgtcagcggtggaccgtggaggccacctaccggaacatgactgagaagcaagcgctaagctggggcctgggccaccacgcattttgccggaacccagataatgacacacgtccatggtgcttcgtctggagtggcgacaggctgagctgggactattgcggcctggagcagtgccagacgccaacgtttgcacctctagttgtccctgagagtcaggaggagtccccgtcccaggcaccatctctgtcccatgcaccaaatgactcgaccgatcatcagacttctctgtccaagaccaacacgatgggctgcggacagaggttccgcaagggactgtcctcgttcatgcgcgtggtgggcggactagtggctctgcctgggtcgcacccctacatcgctgcactgtactggggtaacaacttctgcgcgggcagtctcatcgccccctgttgggtgctgaccgcggctcactgcctgcagaatcggccagcgcccgaggaactgacagtggtacttggtcaagatcgccacaaccagagctgcgagtggtgccagactctggctgtgcgctcctaccgccttcacgagggcttctcctccatcacctaccagcacgacttggctctgctgcgcctgcaggaaagcaaaaccaacagttgcgcgatcctgtcacctcacgttcagcctgtgtgtctacccagcggcgcggccccaccctctgagacagtgctctgcgaggtggccggctggggtcaccagttcgagggggctgaagaatactccaccttcctgcaggaggcacaggttccctttatcgccctggatcgctgctccaactctaacgtgcacggagacgccattctccctgggatgctttgcgctggcttcttggagggaggcaccgatgcctgccagggtgactccgggggccctctggtgtgtgaggaaggaactgcagaacatcagctcaccctgcgcggagtcatcagctggggctccggctgtggtgaccgcaacaagcccggagtctacacagacgtggccaactacctggcttggatccagaagcatattgcttcataa

SEQ ID NO: 10 - DNA, 57 bp, Mus musculus
atgacggctctgttgttcctggggtctctgctgatgagtctggatctgacactttcg

SEQ ID NO: 11 - DNA, 1005 bp, Mus musculus
gctccaccatggaaagactccaagaaatttaaggacgcacctgatgggcccacagtggttctcactgtggatgggaggctctgccattttccctttcagtaccaccgtcagctacaccacaaatgcatccacaaaaggcggccaggctcccgcccctggtgtgctaccacccccaactttgatgaagatcagcaatggggatactgcttggagcccaagaaagtgaaagaccattgcagcaaacacaacccgtgccacaaaggagggacatgtatcaacacccccaatgggccacactgtctctgccctgaacacctcactgggaaacattgccagaaagagaaatgctttgagcctcagcttctcaagttcttccacgagaatgagctatggtttagaacggggccaggaggtgtggccaggtgcgagtgcaaaggttctgaggctcactgcaagccggtggccagccaggcctgcagcatcaatccgtgccttaatgggggcagctgcctcctcgtggaggaccacccactgtgccgttgccctacaggctacactggatatttttgcgacttggacctttgggcgacctgctatgaaggcagggggctcagctaccggggccaggctggaactacgcaatcgggtgcgccatgtcagcggtggaccgtggaggccacctaccggaacatgactgagaagcaagcgctaagctggggcctgggccaccacgcattttgccggaacccagataatgacacacgtccatggtgcttcgtctggagtggcgacaggctgagctgggactattgcggcctggagcagtgccagacgccaacgtttgcacctctagttgtccctgagagtcaggaggagtccccgtcccaggcaccatctctgtcccatgcaccaaatgactcgaccgatcatcagacttctctgtccaagaccaacacgatgggctgcggacagaggttccgcaagggactgtcctcgttcatgcgc

SEQ ID NO: 12 - DNA, 729 bp, Mus musculus
gtggtgggcggactagtggctctgcctgggtcgcacccctacatcgctgcactgtactggggtaacaacttctgcgcgggcagtctcatcgccccctgttgggtgctgaccgcggctcactgcctgcagaatcggccagcgcccgaggaactgacagtggtacttggtcaagatcgccacaaccagagctgcgagtggtgccagactctggctgtgcgctcctaccgccttcacgagggcttctcctccatcacctaccagcacgacttggctctgctgcgcctgcaggaaagcaaaaccaacagttgcgcgatcctgtcacctcacgttcagcctgtgtgtctacccagcggcgcggccccaccctctgagacagtgctctgcgaggtggccggctggggtcaccagttcgagggggctgaagaatactccaccttcctgcaggaggcacaggttccctttatcgccctggatcgctgctccaactctaacgtgcacggagacgccattctccctgggatgctttgcgctggcttcttggagggaggcaccgatgcctgccagggtgactccgggggccctctggtgtgtgaggaaggaactgcagaacatcagctcaccctgcgcggagtcatcagctggggctccggctgtggtgaccgcaacaagcccggagtctacacagacgtggccaactacctggcttggatccagaagcatattgcttca

SEQ ID NO: 13 - DNA, 1848 bp, Homo sapiens
  misc_feature (1)..(57): Signal Peptide
  misc_feature (58)..(1116): Heavy Chain
  misc_feature (1117)..(1845): Light Chain
atgagggctctgctgctcctggggttcctgctggtgagcttggagtcaacactttcgattccaccttgggaagcccccaaggagcataagtacaaagctgaagagcacacagtcgttctcactgtcaccggggagccctgccacttccccttccagtaccaccggcagctgtaccacaaatgtacccacaagggccggccaggccctcagccctggtgtgctaccacccccaactttgatcaggaccagcgatggggatactgtttggagcccaagaaagtgaaagaccactgcagcaaacacagcccctgccagaaaggagggacctgtgtgaacatgccaagcggcccccactgtctctgtccacaacacctcactggaaaccactgccagaaagagaagtgctttgagcctcagcttctccggtttttccacaagaatgagatatggtatagaactgagcaagcagctgtggccagatgccagtgcaagggtcctgatgcccactgccagcggctggccagccaggcctgccgcaccaacccgtgcctccatgggggtcgctgcctagaggtggagggccaccgcctgtgccactgcccggtgggctacaccggacccttctgcgacgtggacaccaaggcaagctgctatgatggccgcgggctcagctaccgcggcctggccaggaccacgctctcgggtgcgccctgtcagccgtgggcctcggaggccacctaccggaacgtgactgccgagcaagcgcggaactggggactgggcggccacgccttctgccggaacccggacaacgacatccgcccgtggtgcttcgtgctgaaccgcgaccggctgagctgggagtactgcgacctggcacagtgccagaccccaacccaggcggcgcctccgaccccggtgtcccctaggcttcatgtcccactcatgcccgcgcagccggcaccgccgaagcctcagcccacgacccggaccccgcctcagtcccagaccccgggagccttgccggcgaagcgggagcagccgccttccctgaccaggaacggcccactgagctgcgggcagcggctccgcaagagtctgtcttcgatgacccgcgtcgttggcgggctggtggcgctacgcggggcgcacccctacatcgccgcgctgtactggggccacagtttctgcgccggcagcctcatcgccccctgctgggtgctgacggccgctcactgcctgcaggaccggcccgcacccgaggatctgacggtggtgctcggccaggaacgccgtaaccacagctgtgagccgtgccagacgttggccgtgcgctcctaccgcttgcacgaggccttctcgcccgtcagctaccagcacgacctggctctgttgcgccttcaggaggatgcggacggcagctgcgcgctcctgtcgccttacgttcagccggtgtgcctgccaagcggcgccgcgcgaccctccgagaccacgctctgccaggtggccggctggggccaccagttcgagggggcggaggaatatgccagcttcctgcaggaggcgcaggtaccgttcctctccctggagcgctgctcagccccggacgtgcacggatcctccatcctccccggcatgctctgcgcagggttcctcgagggcggcaccgatgcgtgccagggtgattccggaggcccgctggtgtgtgaggaccaagctgcagagcgccggctcaccctgcaaggcatcatcagctggggatcgggctgtggtgaccgcaacaagccaggcgtctacaccgatgtggcctactacctggcctggatccgggagcacaccgtttcctga

SEQ ID NO: 14 - DNA, 57 bp, Homo sapiens
atgagggctctgctgctcctggggttcctgctggtgagcttggagtcaacactttcg

SEQ ID NO: 15 - DNA, 1059 bp, Homo sapiens
attccaccttgggaagcccccaaggagcataagtacaaagctgaagagcacacagtcgttctcactgtcaccggggagccctgccacttccccttccagtaccaccggcagctgtaccacaaatgtacccacaagggccggccaggccctcagccctggtgtgctaccacccccaactttgatcaggaccagcgatggggatactgtttggagcccaagaaagtgaaagaccactgcagcaaacacagcccctgccagaaaggagggacctgtgtgaacatgccaagcggcccccactgtctctgtccacaacacctcactggaaaccactgccagaaagagaagtgctttgagcctcagcttctccggtttttccacaagaatgagatatggtatagaactgagcaagcagctgtggccagatgccagtgcaagggtcctgatgcccactgccagcggctggccagccaggcctgccgcaccaacccgtgcctccatgggggtcgctgcctagaggtggagggccaccgcctgtgccactgcccggtgggctacaccggacccttctgcgacgtggacaccaaggcaagctgctatgatggccgcgggctcagctaccgcggcctggccaggaccacgctctcgggtgcgccctgtcagccgtgggcctcggaggccacctaccggaacgtgactgccgagcaagcgcggaactggggactgggcggccacgccttctgccggaacccggacaacgacatccgcccgtggtgcttcgtgctgaaccgcgaccggctgagctgggagtactgcgacctggcacagtgccagaccccaacccaggcggcgcctccgaccccggtgtcccctaggcttcatgtcccactcatgcccgcgcagccggcaccgccgaagcctcagcccacgacccggaccccgcctcagtcccagaccccgggagccttgccggcgaagcgggagcagccgccttccctgaccaggaacggcccactgagctgcgggcagcggctccgcaagagtctgtcttcgatgacccgc

SEQ ID NO: 16 - DNA, 729 bp, Homo sapiens
gtcgttggcgggctggtggcgctacgcggggcgcacccctacatcgccgcgctgtactggggccacagtttctgcgccggcagcctcatcgccccctgctgggtgctgacggccgctcactgcctgcaggaccggcccgcacccgaggatctgacggtggtgctcggccaggaacgccgtaaccacagctgtgagccgtgccagacgttggccgtgcgctcctaccgcttgcacgaggccttctcgcccgtcagctaccagcacgacctggctctgttgcgccttcaggaggatgcggacggcagctgcgcgctcctgtcgccttacgttcagccggtgtgcctgccaagcggcgccgcgcgaccctccgagaccacgctctgccaggtggccggctggggccaccagttcgagggggcggaggaatatgccagcttcctgcaggaggcgcaggtaccgttcctctccctggagcgctgctcagccccggacgtgcacggatcctccatcctccccggcatgctctgcgcagggttcctcgagggcggcaccgatgcgtgccagggtgattccggaggcccgctggtgtgtgaggaccaagctgcagagcgccggctcaccctgcaaggcatcatcagctggggatcgggctgtggtgaccgcaacaagccaggcgtctacaccgatgtggcctactacctggcctggatccgggagcacaccgtttcc

SEQ ID NO: 17 - DNA, 12176 bp, Artificial Sequence
  Synthetic
  misc_feature (1)..(19): Mouse Sequence
  misc_feature (20)..(3893): Human Sequence
  misc_feature (20)..(22): Start Codon
  misc_feature (3742)..(3812): Exon 4
  misc_feature (3894)..(8703): Neo Self-Deleting Cassette
  misc_feature (3894)..(3899): XhoI
  misc_feature (3900)..(3933): LoxP
  misc_feature (8632)..(8665): LoxP
  misc_feature (8672)..(8697): I_Ceu
  misc_feature (8698)..(8703): NheI
  misc_feature (8704)..(12065): Human Sequence
  misc_feature (8924)..(9034): Exon 5
  misc_feature (9172)..(9303): Exon 6
  misc_feature (9443)..(9547): Exon 7
  misc_feature (12063)..(12065): Stop Codon
  misc_feature (12066)..(12176): Mouse Sequence
ggggccatcggcagacgccatgagggctctgctgctcctggggttcctgctggtgagcttggagtcaacactttcggtgagtgctgtgggaaccaggattgtcccaggattgttctggggggtcgctatcacagccatgagccatggcctctgctcatgacctgtgggtccaggtgactaggaggcctatgtggaaaggtgaggccagcccggaaggcccaggcagaggagacagacaaccagactgggtggatacaagggcacagcctgcatttctgggggagatgggccttaagaagacaacggggggaggtagaaagggtttgggtcttgggaagaaatctctgcatttctgggctgtgagaggaagctgcagactagcaacagatcggtggcaggctatgacttatagtcagttccctgccttcttctctcccttgtagattccaccttgggaagcccccaaggagcataagtacaaagctgaagagcacacagtcggtaagtggcctggctcctcctcccgggaacccttgggtggggatgtgtatggtgcagtgtgtgcagtctcagggcagtctagtctagtgcctacctggtgctaggtcttatgcccatgggcactagagtgatcgtgagctgtgtgatccttgagggcagggtatgggctgtgtctaagtgcccacgagcctggctcggagcaggtgcttgagatatgtgctgctggcgccatcacacctgggctcctgccagccttcctcagtttccccagcttctccccttcttttcctttccccagtacgtctcatgggcatcattcatgccacacagaggccagggccttcaatgggcaaggaaggatcaagagcttgtctctggcatctgaatgcctctgaagcccagctttatcacttatgagctgggtgactctgggcgagggatttgagttctccaagcttcaatttccccttctgtgaaaccaggttgataacagtaaacctcttagggttgttgagaagggaaacccatgtgaggtattcagcccatcacctggtgcatggaaatgctttacaaatattagcttttattatgaaactaccttttagatgaagggtacctgccatttcccccttcctcaagctctgccatagctccccattgctttcattcttccagacactaaattacctacatgccaggcatggtggctcatgcctgtaatcccagcactttgggaggccaaggtcggtggatcatgaggtcaggagttcgagaccagcctggccaacatggtgaaatgctgtctctactaaaagtacaaaaattagccaggcatggtggcatgcgccagtagtcccagctactcgggaggctgaggcagaagaattgcttgaacctgggaggtgaaggttgcagtgaacgaagatcacaccattgcactccagcttgggcaacacagcaagactccgtctcaaaaaaaaaaaaaaaatttacctagagtgtggcacatagcagggcctgtgaaccagatggaccttaccctggtgggcctgacttggtggggttgagtctctaagcatggcgttgaggcccagcacattccaaccctggactccctcagcctcctctcttcaccccacacccaaaagtttctcctctctcttgccttacccaaacttggtgccctatccttgcctaatcccctgcctaaggtccccctcctctctgtccgtccatcccatctgcatctttttttttttttgagatggagtctcgctctgtcccctaggctagagtgcaatggcgcgatcttggctcattgcaacctccgcctcctgggttcaagcgattctctgcctcagcctcccgagttgctgggattacaggcacacaacttcatgctcagctaatttttgtattttttagtagagacagggtttcaccatgttggccaggctggtctcgaactcctgccctcaggtggtccgcccaccttagcctcccaaagtgctgggattacaggcgtgagccaccgcgcctggcccccatttgcatcttaaaggtccatctcagatccatttccatttactgtcctagttctggtttggtccttggcaagtgcactttgccttgaacaaaatagtggcaaaagcttattgagcaggtactttgtgccagacactgctcagcatttcatggcattatctcatgaagccccacgacaattcctctgaagaagacacaggcaattctcattattcgcgatggttatgttctataaaatcacagtgaacattgaactagcaaacagtattaggttcctgtgagcctctggtcacaacattttcatcaaccaacagcatataatctggttttatgtatgattctgtttaaagacattttatttagtatatgtgttgctgattcatcaatgctaagctgatggcactatagcacacacctgaatcaagtgtctaacacacgctttctccctaaggtagccttcttgtgcttaggaactacacagctcttcagcaggaggctcagaggccatttccaaaagccaaatccccagcaaaagcacaaagtgtgaaaaacgttgcactaagtagactgagaaggacactcattcaataggagagctgaaacaagcagcagcagcgtgacgccttgttgaaccttaactgggaatgtgcaaatttttcactgctctgtgcatgcccacaaatggccatgaaaacatttcaagtattgacttgggagttacaaataaaattcagcaagtaggcacattctcaatgtagaaccagagaagaatgaggatcaactgtactattattactgccgttttacagataaggaaaccaaggctcagatcagagtggttaacagtgacttcaacattcaacaagtattattaagtgcctactttgtggcaagtgctcttcctggccttgggactgaagacttacccaaggtcacacagctagcaggttgtggagtcaggagtctactccagctatctgactcctgaacccaagtttttttttttttctttaagatggagtctcactctgtcacccaggctggagtgcagtggcgcgatctcggctcactgcaagctccgcctcccgggttcacaccattctcctgcctcggcctcccgagtagctgggactacaggcacctgccaccacccccagctaatttttttgtatttttagtagagagggggtttcactgtattagccaggatggtcttgatctcctgacctcgtgatctgcccgccttggcctcccaaagtgctgggattacaggcttgagccaccgcgcccggccctgaacccaacttttagagcagaaagtgttttcaatgcacagcgacctttttgagggtctgtccttttcctgaccagaccctgagggacagtgcctgagcagttgagtacaggggaagtcctcagagagtgtgttgtccctgcagttctcactgtcaccggggagccctgccacttccccttccagtaccaccggcagctgtaccacaaatgtacccacaagggccggccaggccctcagccctggtaagactacgcagaggagttggagcaggggcctgggagacatgtaccctgcctgtccttctgtccaaggaactctgcttggagagaggggactgtgatagggcagggtgggccaggcccctgggtagagcagggaagccttgtctctttctacaggtgtgctaccacccccaactttgatcaggaccagcgatggggatactgtttggagcccaagaaagtgaaaggtgctacacacagcctctggggtggcctggggctctctcctcccgcctcattactctcctggtatcaccagaccccacacactcgagataacttcgtataatgtatgctatacgaagttatatgcatgccagtagcagcacccacgtccaccttctgtctagtaatgtccaacacctccctcagtccaaacactgctctgcatccatgtggctcccatttatacctgaagcacttgatggggcctcaatgttttactagagcccacccccctgcaactctgagaccctctggatttgtctgtcagtgcctcactggggcgttggataatttcttaaaaggtcaagttccctcagcagcattctctgagcagtctgaagatgtgtgcttttcacagttcaaatccatgtggctgtttcacccacctgcctggccttgggttatctatcaggacctagcctagaagcaggtgtgtggcacttaacacctaagctgagtgactaactgaacactcaagtggatgccatctttgtcacttcttgactgtgacacaagcaactcctgatgccaaagccctgcccacccctctcatgcccatatttggacatggtacaggtcctcactggccatggtctgtgaggtcctggtcctctttgacttcataattcctaggggccactagtatctataagaggaagagggtgctggctcccaggccacagcccacaaaattccacctgctcacaggttggctggctcgacccaggtggtgtcccctgctctgagccagctcccggccaagccagcaccatgggaacccccaagaagaagaggaaggtgcgtaccgatttaaattccaatttactgaccgtacaccaaaatttgcctgcattaccggtcgatgcaacgagtgatgaggttcgcaagaacctgatggacatgttcagggatcgccaggcgttttctgagcatacctggaaaatgcttctgtccgtttgccggtcgtgggcggcatggtgcaagttgaataaccggaaatggtttcccgcagaacctgaagatgttcgcgattatcttctatatcttcaggcgcgcggtctggcagtaaaaactatccagcaacatttgggccagctaaacatgcttcatcgtcggtccgggctgccacgaccaagtgacagcaatgctgtttcactggttatgcggcggatccgaaaagaaaacgttgatgccggtgaacgtgcaaaacaggtaaatataaaatttttaagtgtataatgatgttaaactactgattctaattgtttgtgtattttaggctctagcgttcgaacgcactgatttcgaccaggttcgttcactcatggaaaatagcgatcgctgccaggatatacgtaatctggcatttctggggattgcttataacaccctgttacgtatagccgaaattgccaggatcagggttaaagatatctcacgtactgacggtgggagaatgttaatccatattggcagaacgaaaacgctggttagcaccgcaggtgtagagaaggcacttagcctgggggtaactaaactggtcgagcgatggatttccgtctctggtgtagctgatgatccgaataactacctgttttgccgggtcagaaaaaatggtgttgccgcgccatctgccaccagccagctatcaactcgcgccctggaagggatttttgaagcaactcatcgattgatttacggcgctaaggatgactctggtcagagatacctggcctggtctggacacagtgcccgtgtcggagccgcgcgagatatggcccgcgctggagtttcaataccggagatcatgcaagctggtggctggaccaatgtaaatattgtcatgaactatatccgtaacctggatagtgaaacaggggcaatggtgcgcctgctggaagatggcgattaggcggccggccgctaatcagccataccacatttgtagaggttttacttgctttaaaaaacctcccacacctccccctgaacctgaaacataaaatgaatgcaattgttgttgttaacttgtttattgcagcttataatggttacaaataaagcaatagcatcacaaatttcacaaataaagcatttttttcactgcattctagttgtggtttgtccaaactcatcaatgtatcttatcatgtctggatcccccggctagagtttaaacactagaactagtggatcccccgggatcatggcctccgcgccgggttttggcgcctcccgcgggcgcccccctcctcacggcgagcgctgccacgtcagacgaagggcgcagcgagcgtcctgatccttccgcccggacgctcaggacagcggcccgctgctcataagactcggccttagaaccccagtatcagcagaaggacattttaggacgggacttgggtgactctagggcactggttttctttccagagagcggaacaggcgaggaaaagtagtcccttctcggcgattctgcggagggatctccgtggggcggtgaacgccgatgattatataaggacgcgccgggtgtggcacagctagttccgtcgcagccgggatttgggtcgcggttcttgtttgtggatcgctgtgatcgtcacttggtgagtagcgggctgctgggctggccggggctttcgtggccgccgggccgctcggtgggacggaagcgtgtggagagaccgccaagggctgtagtctgggtccgcgagcaaggttgccctgaactgggggttggggggagcgcagcaaaatggcggctgttcccgagtcttgaatggaagacgcttgtgaggcgggctgtgaggtcgttgaaacaaggtggggggcatggtgggcggcaagaacccaaggtcttgaggccttcgctaatgcgggaaagctcttattcgggtgagatgggctggggcaccatctggggaccctgacgtgaagtttgtcactgactggagaactcggtttgtcgtctgttgcgggggcggcagttatggcggtgccgttgggcagtgcacccgtacctttgggagcgcgcgccctcgtcgtgtcgtgacgtcacccgttctgttggcttataatgcagggtggggccacctgccggtaggtgtgcggtaggcttttctccgtcgcaggacgcagggttcgggcctagggtaggctctcctgaatcgacaggcgccggacctctggtgaggggagggataagtgaggcgtcagtttctttggtcggttttatgtacctatcttcttaagtagctgaagctccggttttgaactatgcgctcggggttggcgagtgtgttttgtgaagttttttaggcaccttttgaaatgtaatcatttgggtcaatatgtaattttcagtgttagactagtaaattgtccgctaaattctggccgtttttggcttttttgttagacgtgttgacaattaatcatcggcatagtatatcggcatagtataatacgacaaggtgaggaactaaaccatgggatcggccattgaacaagatggattgcacgcaggttctccggccgcttgggtggagaggctattcggctatgactgggcacaacagacaatcggctgctctgatgccgccgtgttccggctgtcagcgcaggggcgcccggttctttttgtcaagaccgacctgtccggtgccctgaatgaactgcaggacgaggcagcgcggctatcgtggctggccacgacgggcgttccttgcgcagctgtgctcgacgttgtcactgaagcgggaagggactggctgctattgggcgaagtgccggggcaggatctcctgtcatctcaccttgctcctgccgagaaagtatccatcatggctgatgcaatgcggcggctgcatacgcttgatccggctacctgcccattcgaccaccaagcgaaacatcgcatcgagcgagcacgtactcggatggaagccggtcttgtcgatcaggatgatctggacgaagagcatcaggggctcgcgccagccgaactgttcgccaggctcaaggcgcgcatgcccgacggcgatgatctcgtcgtgacccatggcgatgcctgcttgccgaatatcatggtggaaaatggccgcttttctggattcatcgactgtggccggctgggtgtggcggaccgctatcaggacatagcgttggctacccgtgatattgctgaagagcttggcggcgaatgggctgaccgcttcctcgtgctttacggtatcgccgctcccgattcgcagcgcatcgccttctatcgccttcttgacgagttcttctgaggggatccgctgtaagtctgcagaaattgatgatctattaaacaataaagatgtccactaaaatggaagtttttcctgtcatactttgttaagaagggtgagaacagagtacctacattttgaatggaaggattggagctacgggggtgggggtggggtgggattagataaatgcctgctctttactgaaggctctttactattgctttatgataatgtttcatagttggatatcataatttaaacaagcaaaaccaaattaagggccagctcattcctcccactcatgatctatagatctatagatctctcgtgggatcattgtttttctcttgattcccactttgtggttctaagtactgtggtttccaaatgtgtcagtttcatagcctgaagaacgagatcagcagcctctgttccacatacacttcattctcagtattgttttgccaagttctaattccatcagacctcgacctgcagcccctagataacttcgtataatgtatgctatacgaagttatgctaggtaactataacggtcctaaggtagcgagctagccctgggattctggacccagccccttctctccctccacaataccctttggaagtccagagggagagttctgggaaggagtggtcccattttgcaggtgggtaaaccaagcttggaaacttggagtagcaaggtcacaaggcaagtaggttcaagaagggccttggcccccagctgtgtgactcagctccctgctcttccttccaccatgtccatctctcagaccactgcagcaaacacagcccctgccagaaaggagggacctgtgtgaacatgccaagcggcccccactgtctctgtccacaacacctcactggaaaccactgccagaaaggtgaggagatgtggaggacctgggcggggtgctgggggacaggggcaaccctgggcctacagaataggttgctggatactcggagacttggcatggtcctagactctcctgagaccactatccctctttgtccccagagaagtgctttgagcctcagcttctccggtttttccacaagaatgagatatggtatagaactgagcaagcagctgtggccagatgccagtgcaagggtcctgatgcccactgccagcggctggccagccagggtgagcagatggttgggaacgggccagggaggagcgtcaggaagacaggctggcaggaggccgggtggtgtgccaggaaggagagctctctgggggggtctttaggcccaggggtggctcactgcgttccctccccaagcctgccgcaccaacccgtgcctccatgggggtcgctgcctagaggtggagggccaccgcctgtgccactgcccggtgggctacaccggacccttctgcgacgtgggtgagtgagggtctggggcaagcagaaggccagcccccaggtgggacgggcttgccaggaaggaggagggagagtgcggaaagcagatgagagggaggcaggagagcccagccttggctgcccagggagccccctttctcctcagacaccaaggcaagctgctatgatggccgcgggctcagctaccgcggcctggccaggaccacgctctcgggtgcgccctgtcagccgtgggcctcggaggccacctaccggaacgtgactgccgagcaagcgcggaactggggactgggcggccacgccttctgccggtgcgccgcgtggggctgggtgacccctccgccccagggctccgggctcccggcgctctaacggcgccccgtcgtgtggctacaggaacccggacaacgacatccgcccgtggtgcttcgtgctgaaccgcgaccggctgagctgggagtactgcgacctggcacagtgccagaccccaacccaggcggcgcctccgaccccggtgtcccctaggcttcatgtcccactcatgcccgcgcagccggcaccgccgaagcctcagcccacgacccggaccccgcctcagtcccagaccccgggaggttaggaagtgggggggggaaggaggagccgagagggcgccgggcgagctagattccggccagccggccgcgggctctccgtcctcagcccctgctcctccacagccttgccggcgaagcgggagcagccgccttccctgaccaggaacggcccactgagctgcgggcagcggctccgcaagagtctgtcttcgatgacccgcgtcgttggcgggctggtggcgctacgcggggcgcacccctacatcgccgcgctgtactggggccacagtttctgcgccggcagcctcatcgccccctgctgggtgctgacggccgctcactgcctgcaggaccggcgagtacccgcccgcccagagccgccccaggggccgcggctcctccgtctcccagcgcagcttccacgctgcacccgaacccgtgccctaccttctcccgccccacccttctttccacgcccctccggagctcccggggaggaagctggaacacgggattggggttcgggagcagggggcttccccagaacgcttgtggccaggtctgagagcgctgcctctcccctaccccccccgcaggcccgcacccgaggatctgacggtggtgctcggccaggaacgccgtaaccacagctgtgagccgtgccagacgttggccgtgcgctcctaccgcttgcacgaggccttctcgcccgtcagctaccagcacgacctgggtgcgtgggggcgccccgcggggacgggaagagagcttggggccccggcgtccccgcctcacgctcctctccgcccgggttagctctgttgcgccttcaggaggatgcggacggcagctgcgcgctcctgtcgccttacgttcagccggtgtgcctgccaagcggcgccgcgcgaccctccgagaccacgctctgccaggtggccggctggggccaccagttcgagggtaggcacaactgctaggggcaggggtaggggaggagacctttgatcactgggttaggcggaagaagcccgcgactttggtatcgttccgggtgcctacagaatgggtggcgctgacctgatgggttgtgagaatgtgtaggtgaatcccaggtagaatcccagggcctgggattcactgctgggatccccaaatctcctggggatacagggagaatcgaacttgctcttggttccctctgggcgccgggctgcaaaggccaactaggacgctggccccgcgctccgggctagtgtgggagccaggttctgcgactctggatgggtggtgggggaggggtttctgtttccgctccgcccattcaaatcctggcttttctctggacctcagcctccttgcctatgaaattgaattaatggcacctcctccccttcgggcttgctgcgagagaggaagggcatgagtgggtttacaagcgcctggagcagctttgtccatcgtccgggcggcaagcgttgtcagatggggtgtgaagaaggcgctctgtgttcgcaggggcggaggaatatgccagcttcctgcaggaggcgcaggtaccgttcctctccctggagcgctgctcagccccggacgtgcacggatcctccatcctccccggcatgctctgcgcagggttcctcgagggcggcaccgatgcgtgccaggtgagctcttagcccggttggcgcccttccccgaggccgtcaggcacaaatctcaggtccacagcgctgagctgcgtgtttccgacccagggtgattccggaggcccgctggtgtgtgaggaccaagctgcagagcgccggctcaccctgcaaggcatcatcagctggggatcgggctgtggtgaccgcaacaagccaggcgtctacaccgatgtggcctactacctggcctggatccgggagcacaccgtttcctgactaaccaggctttatccttccctccttgtgtgctccttgggatgggacgatgaatgtggcatgctgggtcacagtgaagctagtgccccgacactgggggcacagaaactc

SEQ ID NO: 18 - DNA, 7444 bp, Artificial Sequence
  Synthetic
  misc_feature (1)..(19): Mouse Sequence
  misc_feature (20)..(3893): Human Sequence
  misc_feature (20)..(22): Start Codon
  misc_feature (3742)..(3812): Exon 4
  misc_feature (3894)..(3971): Deleted Neo Self-Deleting Cassette
  misc_feature (3894)..(3899): XhoI
  misc_feature (3900)..(3933): LoxP
  misc_feature (3940)..(3965): I_Ceu
  misc_feature (3966)..(3971): NheI
  misc_feature (3972)..(7333): Human Sequence
  misc_feature (4192)..(4302): Exon 5
  misc_feature (4440)..(4571): Exon 6
  misc_feature (4711)..(4815): Exon 7
  misc_feature (7331)..(7333): Stop Codon
  misc_feature (7334)..(7444): Mouse Sequence
ggggccatcggcagacgccatgagggctctgctgctcctggggttcctgctggtgagcttggagtcaacactttcggtgagtgctgtgggaaccaggattgtcccaggattgttctggggggtcgctatcacagccatgagccatggcctctgctcatgacctgtgggtccaggtgactaggaggcctatgtggaaaggtgaggccagcccggaaggcccaggcagaggagacagacaaccagactgggtggatacaagggcacagcctgcatttctgggggagatgggccttaagaagacaacggggggaggtagaaagggtttgggtcttgggaagaaatctctgcatttctgggctgtgagaggaagctgcagactagcaacagatcggtggcaggctatgacttatagtcagttccctgccttcttctctcccttgtagattccaccttgggaagcccccaaggagcataagtacaaagctgaagagcacacagtcggtaagtggcctggctcctcctcccgggaacccttgggtggggatgtgtatggtgcagtgtgtgcagtctcagggcagtctagtctagtgcctacctggtgctaggtcttatgcccatgggcactagagtgatcgtgagctgtgtgatccttgagggcagggtatgggctgtgtctaagtgcccacgagcctggctcggagcaggtgcttgagatatgtgctgctggcgccatcacacctgggctcctgccagccttcctcagtttccccagcttctccccttcttttcctttccccagtacgtctcatgggcatcattcatgccacacagaggccagggccttcaatgggcaaggaaggatcaagagcttgtctctggcatctgaatgcctctgaagcccagctttatcacttatgagctgggtgactctgggcgagggatttgagttctccaagcttcaatttccccttctgtgaaaccaggttgataacagtaaacctcttagggttgttgagaagggaaacccatgtgaggtattcagcccatcacctggtgcatggaaatgctttacaaatattagcttttattatgaaactaccttttagatgaagggtacctgccatttcccccttcctcaagctctgccatagctccccattgctttcattcttccagacactaaattacctacatgccaggcatggtggctcatgcctgtaatcccagcactttgggaggccaaggtcggtggatcatgaggtcaggagttcgagaccagcctggccaacatggtgaaatgctgtctctactaaaagtacaaaaattagccaggcatggtggcatgcgccagtagtcccagctactcgggaggctgaggcagaagaattgcttgaacctgggaggtgaaggttgcagtgaacgaagatcacaccattgcactccagcttgggcaacacagcaagactccgtctcaaaaaaaaaaaaaaaatttacctagagtgtggcacatagcagggcctgtgaaccagatggaccttaccctggtgggcctgacttggtggggttgagtctctaagcatggcgttgaggcccagcacattccaaccctggactccctcagcctcctctcttcaccccacacccaaaagtttctcctctctcttgccttacccaaacttggtgccctatccttgcctaatcccctgcctaaggtccccctcctctctgtccgtccatcccatctgcatctttttttttttttgagatggagtctcgctctgtcccctaggctagagtgcaatggcgcgatcttggctcattgcaacctccgcctcctgggttcaagcgattctctgcctcagcctcccgagttgctgggattacaggcacacaacttcatgctcagctaatttttgtattttttagtagagacagggtttcaccatgttggccaggctggtctcgaactcctgccctcaggtggtccgcccaccttagcctcccaaagtgctgggattacaggcgtgagccaccgcgcctggcccccatttgcatcttaaaggtccatctcagatccatttccatttactgtcctagttctggtttggtccttggcaagtgcactttgccttgaacaaaatagtggcaaaagcttattgagcaggtactttgtgccagacactgctcagcatttcatggcattatctcatgaagccccacgacaattcctctgaagaagacacaggcaattctcattattcgcgatggttatgttctataaaatcacagtgaacattgaactagcaaacagtattaggttcctgtgagcctctggtcacaacattttcatcaaccaacagcatataatctggttttatgtatgattctgtttaaagacattttatttagtatatgtgttgctgattcatcaatgctaagctgatggcactatagcacacacctgaatcaagtgtctaacacacgctttctccctaaggtagccttcttgtgcttaggaactacacagctcttcagcaggaggctcagaggccatttccaaaagccaaatccccagcaaaagcacaaagtgtgaaaaacgttgcactaagtagactgagaaggacactcattcaataggagagctgaaacaagcagcagcagcgtgacgccttgttgaaccttaactgggaatgtgcaaatttttcactgctctgtgcatgcccacaaatggccatgaaaacatttcaagtattgacttgggagttacaaataaaattcagcaagtaggcacattctcaatgtagaaccagagaagaatgaggatcaactgtactattattactgccgttttacagataaggaaaccaaggctcagatcagagtggttaacagtgacttcaacattcaacaagtattattaagtgcctactttgtggcaagtgctcttcctggccttgggactgaagacttacccaaggtcacacagctagcaggttgtggagtcaggagtctactccagctatctgactcctgaacccaagtttttttttttttctttaagatggagtctcactctgtcacccaggctggagtgcagtggcgcgatctcggctcactgcaagctccgcctcccgggttcacaccattctcctgcctcggcctcccgagtagctgggactacaggcacctgccaccacccccagctaatttttttgtatttttagtagagagggggtttcactgtattagccaggatggtcttgatctcctgacctcgtgatctgcccgccttggcctcccaaagtgctgggattacaggcttgagccaccgcgcccggccctgaacccaacttttagagcagaaagtgttttcaatgcacagcgacctttttgagggtctgtccttttcctgaccagaccctgagggacagtgcctgagcagttgagtacaggggaagtcctcagagagtgtgttgtccctgcagttctcactgtcaccggggagccctgccacttccccttccagtaccaccggcagctgtaccacaaatgtacccacaagggccggccaggccctcagccctggtaagactacgcagaggagttggagcaggggcctgggagacatgtaccctgcctgtccttctgtccaaggaactctgcttggagagaggggactgtgatagggcagggtgggccaggcccctgggtagagcagggaagccttgtctctttctacaggtgtgctaccacccccaactttgatcaggaccagcgatggggatactgtttggagcccaagaaagtgaaaggtgctacacacagcctctggggtggcctggggctctctcctcccgcctcattactctcctggtatcaccagaccccacacactcgagataacttcgtataatgtatgctatacgaagttatgctaggtaactataacggtcctaaggtagcgagctagccctgggattctggacccagccccttctctccctccacaataccctttggaagtccagagggagagttctgggaaggagtggtcccattttgcaggtgggtaaaccaagcttggaaacttggagtagcaaggtcacaaggcaagtaggttcaagaagggccttggcccccagctgtgtgactcagctccctgctcttccttccaccatgtccatctctcagaccactgcagcaaacacagcccctgccagaaaggagggacctgtgtgaacatgccaagcggcccccactgtctctgtccacaacacctcactggaaaccactgccagaaaggtgaggagatgtggaggacctgggcggggtgctgggggacaggggcaaccctgggcctacagaataggttgctggatactcggagacttggcatggtcctagactctcctgagaccactatccctctttgtccccagagaagtgctttgagcctcagcttctccggtttttccacaagaatgagatatggtatagaactgagcaagcagctgtggccagatgccagtgcaagggtcctgatgcccactgccagcggctggccagccagggtgagcagatggttgggaacgggccagggaggagcgtcaggaagacaggctggcaggaggccgggtggtgtgccaggaaggagagctctctgggggggtctttaggcccaggggtggctcactgcgttccctccccaagcctgccgcaccaacccgtgcctccatgggggtcgctgcctagaggtggagggccaccgcctgtgccactgcccggtgggctacaccggacccttctgcgacgtgggtgagtgagggtctggggcaagcagaaggccagcccccaggtgggacgggcttgccaggaaggaggagggagagtgcggaaagcagatgagagggaggcaggagagcccagccttggctgcccagggagccccctttctcctcagacaccaaggcaagctgctatgatggccgcgggctcagctaccgcggcctggccaggaccacgctctcgggtgcgccctgtcagccgtgggcctcggaggccacctaccggaacgtgactgccgagcaagcgcggaactggggactgggcggccacgccttctgccggtgcgccgcgtggggctgggtgacccctccgccccagggctccgggctcccggcgctctaacggcgccccgtcgtgtggctacaggaacccggacaacgacatccgcccgtggtgcttcgtgctgaaccgcgaccggctgagctgggagtactgcgacctggcacagtgccagaccccaacccaggcggcgcctccgaccccggtgtcccctaggcttcatgtcccactcatgcccgcgcagccggcaccgccgaagcctcagcccacgacccggaccccgcctcagtcccagaccccgggaggttaggaagtgggggggggaaggaggagccgagagggcgccgggcgagctagattccggccagccggccgcgggctctccgtcctcagcccctgctcctccacagccttgccggcgaagcgggagcagccgccttccctgaccaggaacggcccactgagctgcgggcagcggctccgcaagagtctgtcttcgatgacccgcgtcgttggcgggctggtggcgctacgcggggcgcacccctacatcgccgcgctgtactggggccacagtttctgcgccggcagcctcatcgccccctgctgggtgctgacggccgctcactgcctgcaggaccggcgagtacccgcccgcccagagccgccccaggggccgcggctcctccgtctcccagcgcagcttccacgctgcacccgaacccgtgccctaccttctcccgccccacccttctttccacgcccctccggagctcccggggaggaagctggaacacgggattggggttcgggagcagggggcttccccagaacgcttgtggccaggtctgagagcgctgcctctcccctaccccccccgcaggcccgcacccgaggatctgacggtggtgctcggccaggaacgccgtaaccacagctgtgagccgtgccagacgttggccgtgcgctcctaccgcttgcacgaggccttctcgcccgtcagctaccagcacgacctgggtgcgtgggggcgccccgcggggacgggaagagagcttggggccccggcgtccccgcctcacgctcctctccgcccgggttagctctgttgcgccttcaggaggatgcggacggcagctgcgcgctcctgtcgccttacgttcagccggtgtgcctgccaagcggcgccgcgcgaccctccgagaccacgctctgccaggtggccggctggggccaccagttcgagggtaggcacaactgctaggggcaggggtaggggaggagacctttgatcactgggttaggcggaagaagcccgcgactttggtatcgttccgggtgcctacagaatgggtggcgctgacctgatgggttgtgagaatgtgtaggtgaatcccaggtagaatcccagggcctgggattcactgctgggatccccaaatctcctggggatacagggagaatcgaacttgctcttggttccctctgggcgccgggctgcaaaggccaactaggacgctggccccgcgctccgggctagtgtgggagccaggttctgcgactctggatgggtggtgggggaggggtttctgtttccgctccgcccattcaaatcctggcttttctctggacctcagcctccttgcctatgaaattgaattaatggcacctcctccccttcgggcttgctgcgagagaggaagggcatgagtgggtttacaagcgcctggagcagctttgtccatcgtccgggcggcaagcgttgtcagatggggtgtgaagaaggcgctctgtgttcgcaggggcggaggaatatgccagcttcctgcaggaggcgcaggtaccgttcctctccctggagcgctgctcagccccggacgtgcacggatcctccatcctccccggcatgctctgcgcagggttcctcgagggcggcaccgatgcgtgccaggtgagctcttagcccggttggcgcccttccccgaggccgtcaggcacaaatctcaggtccacagcgctgagctgcgtgtttccgacccagggtgattccggaggcccgctggtgtgtgaggaccaagctgcagagcgccggctcaccctgcaaggcatcatcagctggggatcgggctgtggtgaccgcaacaagccaggcgtctacaccgatgtggcctactacctggcctggatccgggagcacaccgtttcctgactaaccaggctttatccttccctccttgtgtgctccttgggatgggacgatgaatgtggcatgctgggtcacagtgaagctagtgccccgacactgggggcacagaaactc

SEQ ID NO: 19 - DNA, 24 bp, Artificial Sequence
  Synthetic
tcggtggcaggctatgacttatag

SEQ ID NO: 20 - DNA, 24 bp, Artificial Sequence
  Synthetic
cagttccctgccttcttctctccc

SEQ ID NO: 21 - DNA, 22 bp, Artificial Sequence
  Synthetic
ggcttcccaaggtggaatctac

SEQ ID NO: 22 - DNA, 23 bp, Artificial Sequence
  Synthetic
aagggcatgagtgggtttacaag

SEQ ID NO: 23 - DNA, 23 bp, Artificial Sequence
  Synthetic
cgcctggagcagctttgtccatc

SEQ ID NO: 24 - DNA, 21 bp, Artificial Sequence
  Synthetic
acacagagcgccttcttcaca

SEQ ID NO: 25 - DNA, 21 bp, Artificial Sequence
  Synthetic
gttcctgccttctctctccta

SEQ ID NO: 26 - DNA, 25 bp, Artificial Sequence
  Synthetic
taggctccaccatggaaagactcca

SEQ ID NO: 27 - DNA, 19 bp, Artificial Sequence
  Synthetic
cccatcaggtgcgtcctta

SEQ ID NO: 28 - DNA, 20 bp, Artificial Sequence
  Synthetic
tcgctgctccaactctaacg

SEQ ID NO: 29 - DNA, 23 bp, Artificial Sequence
  Synthetic
acgccattctccctgggatgctt

SEQ ID NO: 30 - DNA, 22 bp, Artificial Sequence
  Synthetic
atcggtgcctccctccaagaag

SEQ ID NO: 31 - DNA, 3874 bp, Homo sapiens
atgagggctctgctgctcctggggttcctgctggtgagcttggagtcaacactttcggtgagtgctgtgggaaccaggattgtcccaggattgttctggggggtcgctatcacagccatgagccatggcctctgctcatgacctgtgggtccaggtgactaggaggcctatgtggaaaggtgaggccagcccggaaggcccaggcagaggagacagacaaccagactgggtggatacaagggcacagcctgcatttctgggggagatgggccttaagaagacaacggggggaggtagaaagggtttgggtcttgggaagaaatctctgcatttctgggctgtgagaggaagctgcagactagcaacagatcggtggcaggctatgacttatagtcagttccctgccttcttctctcccttgtagattccaccttgggaagcccccaaggagcataagtacaaagctgaagagcacacagtcggtaagtggcctggctcctcctcccgggaacccttgggtggggatgtgtatggtgcagtgtgtgcagtctcagggcagtctagtctagtgcctacctggtgctaggtcttatgcccatgggcactagagtgatcgtgagctgtgtgatccttgagggcagggtatgggctgtgtctaagtgcccacgagcctggctcggagcaggtgcttgagatatgtgctgctggcgccatcacacctgggctcctgccagccttcctcagtttccccagcttctccccttcttttcctttccccagtacgtctcatgggcatcattcatgccacacagaggccagggccttcaatgggcaaggaaggatcaagagcttgtctctggcatctgaatgcctctgaagcccagctttatcacttatgagctgggtgactctgggcgagggatttgagttctccaagcttcaatttccccttctgtgaaaccaggttgataacagtaaacctcttagggttgttgagaagggaaacccatgtgaggtattcagcccatcacctggtgcatggaaatgctttacaaatattagcttttattatgaaactaccttttagatgaagggtacctgccatttcccccttcctcaagctctgccatagctccccattgctttcattcttccagacactaaattacctacatgccaggcatggtggctcatgcctgtaatcccagcactttgggaggccaaggtcggtggatcatgaggtcaggagttcgagaccagcctggccaacatggtgaaatgctgtctctactaaaagtacaaaaattagccaggcatggtggcatgcgccagtagtcccagctactcgggaggctgaggcagaagaattgcttgaacctgggaggtgaaggttgcagtgaacgaagatcacaccattgcactccagcttgggcaacacagcaagactccgtctcaaaaaaaaaaaaaaaatttacctagagtgtggcacatagcagggcctgtgaaccagatggaccttaccctggtgggcctgacttggtggggttgagtctctaagcatggcgttgaggcccagcacattccaaccctggactccctcagcctcctctcttcaccccacacccaaaagtttctcctctctcttgccttacccaaacttggtgccctatccttgcctaatcccctgcctaaggtccccctcctctctgtccgtccatcccatctgcatctttttttttttttgagatggagtctcgctctgtcccctaggctagagtgcaatggcgcgatcttggctcattgcaacctccgcctcctgggttcaagcgattctctgcctcagcctcccgagttgctgggattacaggcacacaacttcatgctcagctaatttttgtattttttagtagagacagggtttcaccatgttggccaggctggtctcgaactcctgccctcaggtggtccgcccaccttagcctcccaaagtgctgggattacaggcgtgagccaccgcgcctggcccccatttgcatcttaaaggtccatctcagatccatttccatttactgtcctagttctggtttggtccttggcaagtgcactttgccttgaacaaaatagtggcaaaagcttattgagcaggtactttgtgccagacactgctcagcatttcatggcattatctcatgaagccccacgacaattcctctgaagaagacacaggcaattctcattattcgcgatggttatgttctataaaatcacagtgaacattgaactagcaaacagtattaggttcctgtgagcctctggtcacaacattttcatcaaccaacagcatataatctggttttatgtatgattctgtttaaagacattttatttagtatatgtgttgctgattcatcaatgctaagctgatggcactatagcacacacctgaatcaagtgtctaacacacgctttctccctaaggtagccttcttgtgcttaggaactacacagctcttcagcaggaggctcagaggccatttccaaaagccaaatccccagcaaaagcacaaagtgtgaaaaacgttgcactaagtagactgagaaggacactcattcaataggagagctgaaacaagcagcagcagcgtgacgccttgttgaaccttaactgggaatgtgcaaatttttcactgctctgtgcatgcccacaaatggccatgaaaacatttcaagtattgacttgggagttacaaataaaattcagcaagtaggcacattctcaatgtagaaccagagaagaatgaggatcaactgtactattattactgccgttttacagataaggaaaccaaggctcagatcagagtggttaacagtgacttcaacattcaacaagtattattaagtgcctactttgtggcaagtgctcttcctggccttgggactgaagacttacccaaggtcacacagctagcaggttgtggagtcaggagtctactccagctatctgactcctgaacccaagtttttttttttttctttaagatggagtctcactctgtcacccaggctggagtgcagtggcgcgatctcggctcactgcaagctccgcctcccgggttcacaccattctcctgcctcggcctcccgagtagctgggactacaggcacctgccaccacccccagctaatttttttgtatttttagtagagagggggtttcactgtattagccaggatggtcttgatctcctgacctcgtgatctgcccgccttggcctcccaaagtgctgggattacaggcttgagccaccgcgcccggccctgaacccaacttttagagcagaaagtgttttcaatgcacagcgacctttttgagggtctgtccttttcctgaccagaccctgagggacagtgcctgagcagttgagtacaggggaagtcctcagagagtgtgttgtccctgcagttctcactgtcaccggggagccctgccacttccccttccagtaccaccggcagctgtaccacaaatgtacccacaagggccggccaggccctcagccctggtaagactacgcagaggagttggagcaggggcctgggagacatgtaccctgcctgtccttctgtccaaggaactctgcttggagagaggggactgtgatagggcagggtgggccaggcccctgggtagagcagggaagccttgtctctttctacaggtgtgctaccacccccaactttgatcaggaccagcgatggggatactgtttggagcccaagaaagtgaaaggtgctacacacagcctctggggtggcctggggctctctcctcccgcctcattactctcctggtatcaccagaccccacaca

SEQ ID NO: 32 - DNA, 3362 bp, Homo sapiens
cctgggattctggacccagccccttctctccctccacaataccctttggaagtccagagggagagttctgggaaggagtggtcccattttgcaggtgggtaaaccaagcttggaaacttggagtagcaaggtcacaaggcaagtaggttcaagaagggccttggcccccagctgtgtgactcagctccctgctcttccttccaccatgtccatctctcagaccactgcagcaaacacagcccctgccagaaaggagggacctgtgtgaacatgccaagcggcccccactgtctctgtccacaacacctcactggaaaccactgccagaaaggtgaggagatgtggaggacctgggcggggtgctgggggacaggggcaaccctgggcctacagaataggttgctggatactcggagacttggcatggtcctagactctcctgagaccactatccctctttgtccccagagaagtgctttgagcctcagcttctccggtttttccacaagaatgagatatggtatagaactgagcaagcagctgtggccagatgccagtgcaagggtcctgatgcccactgccagcggctggccagccagggtgagcagatggttgggaacgggccagggaggagcgtcaggaagacaggctggcaggaggccgggtggtgtgccaggaaggagagctctctgggggggtctttaggcccaggggtggctcactgcgttccctccccaagcctgccgcaccaacccgtgcctccatgggggtcgctgcctagaggtggagggccaccgcctgtgccactgcccggtgggctacaccggacccttctgcgacgtgggtgagtgagggtctggggcaagcagaaggccagcccccaggtgggacgggcttgccaggaaggaggagggagagtgcggaaagcagatgagagggaggcaggagagcccagccttggctgcccagggagccccctttctcctcagacaccaaggcaagctgctatgatggccgcgggctcagctaccgcggcctggccaggaccacgctctcgggtgcgccctgtcagccgtgggcctcggaggccacctaccggaacgtgactgccgagcaagcgcggaactggggactgggcggccacgccttctgccggtgcgccgcgtggggctgggtgacccctccgccccagggctccgggctcccggcgctctaacggcgccccgtcgtgtggctacaggaacccggacaacgacatccgcccgtggtgcttcgtgctgaaccgcgaccggctgagctgggagtactgcgacctggcacagtgccagaccccaacccaggcggcgcctccgaccccggtgtcccctaggcttcatgtcccactcatgcccgcgcagccggcaccgccgaagcctcagcccacgacccggaccccgcctcagtcccagaccccgggaggttaggaagtgggggggggaaggaggagccgagagggcgccgggcgagctagattccggccagccggccgcgggctctccgtcctcagcccctgctcctccacagccttgccggcgaagcgggagcagccgccttccctgaccaggaacggcccactgagctgcgggcagcggctccgcaagagtctgtcttcgatgacccgcgtcgttggcgggctggtggcgctacgcggggcgcacccctacatcgccgcgctgtactggggccacagtttctgcgccggcagcctcatcgccccctgctgggtgctgacggccgctcactgcctgcaggaccggcgagtacccgcccgcccagagccgccccaggggccgcggctcctccgtctcccagcgcagcttccacgctgcacccgaacccgtgccctaccttctcccgccccacccttctttccacgcccctccggagctcccggggaggaagctggaacacgggattggggttcgggagcagggggcttccccagaacgcttgtggccaggtctgagagcgctgcctctcccctaccccccccgcaggcccgcacccgaggatctgacggtggtgctcggccaggaacgccgtaaccacagctgtgagccgtgccagacgttggccgtgcgctcctaccgcttgcacgaggccttctcgcccgtcagctaccagcacgacctgggtgcgtgggggcgccccgcggggacgggaagagagcttggggccccggcgtccccgcctcacgctcctctccgcccgggttagctctgttgcgccttcaggaggatgcggacggcagctgcgcgctcctgtcgccttacgttcagccggtgtgcctgccaagcggcgccgcgcgaccctccgagaccacgctctgccaggtggccggctggggccaccagttcgagggtaggcacaactgctaggggcaggggtaggggaggagacctttgatcactgggttaggcggaagaagcccgcgactttggtatcgttccgggtgcctacagaatgggtggcgctgacctgatgggttgtgagaatgtgtaggtgaatcccaggtagaatcccagggcctgggattcactgctgggatccccaaatctcctggggatacagggagaatcgaacttgctcttggttccctctgggcgccgggctgcaaaggccaactaggacgctggccccgcgctccgggctagtgtgggagccaggttctgcgactctggatgggtggtgggggaggggtttctgtttccgctccgcccattcaaatcctggcttttctctggacctcagcctccttgcctatgaaattgaattaatggcacctcctccccttcgggcttgctgcgagagaggaagggcatgagtgggtttacaagcgcctggagcagctttgtccatcgtccgggcggcaagcgttgtcagatggggtgtgaagaaggcgctctgtgttcgcaggggcggaggaatatgccagcttcctgcaggaggcgcaggtaccgttcctctccctggagcgctgctcagccccggacgtgcacggatcctccatcctccccggcatgctctgcgcagggttcctcgagggcggcaccgatgcgtgccaggtgagctcttagcccggttggcgcccttccccgaggccgtcaggcacaaatctcaggtccacagcgctgagctgcgtgtttccgacccagggtgattccggaggcccgctggtgtgtgaggaccaagctgcagagcgccggctcaccctgcaaggcatcatcagctggggatcgggctgtggtgaccgcaacaagccaggcgtctacaccgatgtggcctactacctggcctggatccgggagcacaccgtttcctga

SEQ ID NO: 33 - DNA, 1971 bp, Mus musculus
actcctgggcaggcagcggggccatcggcagacgccatgacggctctgttgttcctggggtctctgctgatgagtctggatctgacactttcggctccaccatggaaagactccaagaaatttaaggacgcacctgatgggcccacagtggttctcactgtggatgggaggctctgccattttccctttcagtaccaccgtcagctacaccacaaatgcatccacaaaaggcggccaggctcccgcccctggtgtgctaccacccccaactttgatgaagatcagcaatggggatactgcttggagcccaagaaagtgaaagaccattgcagcaaacacaacccgtgccacaaaggagggacatgtatcaacacccccaatgggccacactgtctctgccctgaacacctcactgggaaacattgccagaaagagaaatgctttgagcctcagcttctcaagttcttccacgagaatgagctatggtttagaacggggccaggaggtgtggccaggtgcgagtgcaaaggttctgaggctcactgcaagccggtggccagccaggcctgcagcatcaatccgtgccttaatgggggcagctgcctcctcgtggaggaccacccactgtgccgttgccctacaggctacactggatatttttgcgacttggacctttgggcgacctgctatgaaggcagggggctcagctaccggggccaggctggaactacgcaatcgggtgcgccatgtcagcggtggaccgtggaggccacctaccggaacatgactgagaagcaagcgctaagctggggcctgggccaccacgcattttgccggaacccagataatgacacacgtccatggtgcttcgtctggagtggcgacaggctgagctgggactattgcggcctggagcagtgccagacgccaacgtttgcacctctagttgtccctgagagtcaggaggagtccccgtcccaggcaccatctctgtcccatgcaccaaatgactcgaccgatcatcagacttctctgtccaagaccaacacgatgggctgcggacagaggttccgcaagggactgtcctcgttcatgcgcgtggtgggcggactagtggctctgcctgggtcgcacccctacatcgctgcactgtactggggtaacaacttctgcgcgggcagtctcatcgccccctgttgggtgctgaccgcggctcactgcctgcagaatcggccagcgcccgaggaactgacagtggtacttggtcaagatcgccacaaccagagctgcgagtggtgccagactctggctgtgcgctcctaccgccttcacgagggcttctcctccatcacctaccagcacgacttggctctgctgcgcctgcaggaaagcaaaaccaacagttgcgcgatcctgtcacctcacgttcagcctgtgtgtctacccagcggcgcggccccaccctctgagacagtgctctgcgaggtggccggctggggtcaccagttcgagggggctgaagaatactccaccttcctgcaggaggcacaggttccctttatcgccctggatcgctgctccaactctaacgtgcacggagacgccattctccctgggatgctttgcgctggcttcttggagggaggcaccgatgcctgccagggtgactccgggggccctctggtgtgtgaggaaggaactgcagaacatcagctcaccctgcgcggagtcatcagctggggctccggctgtggtgaccgcaacaagcccggagtctacacagacgtggccaactacctggcttggatccagaagcatattgcttcataactaaccaggctttatccttccctccttgtgtgctccttgggatgggacgatgaatgtggcatgctgggtcacagtgaagctagtgccccgacactgggggcacagaaactcaataaagtgctttgaaaacgttcctcagaa

SEQ ID NO: 34 - DNA, 2060 bp, Homo sapiens
ctattgatctggactcctggataggcagctggaccaacggacggatgccatgagggctctgctgctcctggggttcctgctggtgagcttggagtcaacactttcgattccaccttgggaagcccccaaggagcataagtacaaagctgaagagcacacagtcgttctcactgtcaccggggagccctgccacttccccttccagtaccaccggcagctgtaccacaaatgtacccacaagggccggccaggccctcagccctggtgtgctaccacccccaactttgatcaggaccagcgatggggatactgtttggagcccaagaaagtgaaagaccactgcagcaaacacagcccctgccagaaaggagggacctgtgtgaacatgccaagcggcccccactgtctctgtccacaacacctcactggaaaccactgccagaaagagaagtgctttgagcctcagcttctccggtttttccacaagaatgagatatggtatagaactgagcaagcagctgtggccagatgccagtgcaagggtcctgatgcccactgccagcggctggccagccaggcctgccgcaccaacccgtgcctccatgggggtcgctgcctagaggtggagggccaccgcctgtgccactgcccggtgggctacaccggagccttctgcgacgtggacaccaaggcaagctgctatgatggccgcgggctcagctaccgcggcctggccaggaccacgctctcgggtgcgccctgtcagccgtgggcctcggaggccacctaccggaacgtgactgccgagcaagcgcggaactggggactgggcggccacgccttctgccggaacccggacaacgacatccgcccgtggtgcttcgtgctgaaccgcgaccggctgagctgggagtactgcgacctggcacagtgccagaccccaacccaggcggcgcctccgaccccggtgtcccctaggcttcatgtcccactcatgcccgcgcagccggcaccgccgaagcctcagcccacgacccggaccccgcctcagtcccagaccccgggagccttgccggcgaagcgggagcagccgccttccctgaccaggaacggcccactgagctgcgggcagcggctccgcaagagtctgtcttcgatgacccgcgtcgttggcgggctggtggcgctacgcggggcgcacccctacatcgccgcgctgtactggggccacagtttctgcgccggcagcctcatcgccccctgctgggtgctgacggccgctcactgcctgcaggaccggcccgcacccgaggatctgacggtggtgctcggccaggaacgccgtaaccacagctgtgagccgtgccagacgttggccgtgcgctcctaccgcttgcacgaggccttctcgcccgtcagctaccagcacgacctggctctgttgcgccttcaggaggatgcggacggcagctgcgcgctcctgtcgccttacgttcagccggtgtgcctgccaagcggcgccgcgcgaccctccgagaccacgctctgccaggtggccggctggggccaccagttcgagggggcggaggaatatgccagcttcctgcaggaggcgcaggtaccgttcctctccctggagcgctgctcagccccggacgtgcacggatcctccatcctccccggcatgctctgcgcagggttcctcgagggcggcaccgatgcgtgccagggtgattccggaggcccgctggtgtgtgaggaccaagctgcagagcgccggctcaccctgcaaggcatcatcagctggggatcgggctgtggtgaccgcaacaagccaggcgtctacaccgatgtggcctactacctggcctggatccgggagcacaccgtttcctgattgctcagggactcatctttccctccttggtgattccgcagtgagagagtggctggggcatggaaggcaagattgtgtcccattcccccagtgcggccagctccgcgccaggatggcgcaggaactcaataaagtgctttgaaaatgctgagaaaaaaaaaaa

SEQ ID NO: 35 - protein, 1391 aa, Artificial Sequence
  Synthetic
  MISC_FEATURE (4)..(10): 5' NLS
  MISC_FEATURE (1376)..(1391): 3' NLS
MDKPKKKRKVKYSIGLDIGTNSVGWAVITDEYKVPSKKFKVLGNTDRHSIKKNLIGALLFDSGETAEATRLKRTARRRYTRRKNRICYLQEIFSNEMAKVDDSFFHRLEESFLVEEDKKHERHPIFGNIVDEVAYHEKYPTIYHLRKKLVDSTDKADLRLIYLALAHMIKFRGHFLIEGDLNPDNSDVDKLFIQLVQTYNQLFEENPINASGVDAKAILSARLSKSRRLENLIAQLPGEKKNGLFGNLIALSLGLTPNFKSNFDLAEDAKLQLSKDTYDDDLDNLLAQIGDQYADLFLAAKNLSDAILLSDILRVNTEITKAPLSASMIKRYDEHHQDLTLLKALVRQQLPEKYKEIFFDQSKNGYAGYIDGGASQEEFYKFIKPILEKMDGTEELLVKLNREDLLRKQRTFDNGSIPHQIHLGELHAILRRQEDFYPFLKDNREKIEKILTFRIPYYVGPLARGNSRFAWMTRKSEETITPWNFEEVVDKGASAQSFIERMTNFDKNLPNEKVLPKHSLLYEYFTVYNELTKVKYVTEGMRKPAFLSGEQKKAIVDLLFKTNRKVTVKQLKEDYFKKIECFDSVEISGVEDRFNASLGTYHDLLKIIKDKDFLDNEENEDILEDIVLTLTLFEDREMIEERLKTYAHLFDDKVMKQLKRRRYTGWGRLSRKLINGIRDKQSGKTILDFLKSDGFANRNFMQLIHDDSLTFKEDIQKAQVSGQGDSLHEHIANLAGSPAIKKGILQTVKVVDELVKVMGRHKPENIVIEMARENQTTQKGQKNSRERMKRIEEGIKELGSQILKEHPVENTQLQNEKLYLYYLQNGRDMYVDQELDINRLSDYDVDHIVPQSFLKDDSIDNKVLTRSDKNRGKSDNVPSEEVVKKMKNYWRQLLNAKLITQRKFDNLTKAERGGLSELDKAGFIKRQLVETRQITKHVAQILDSRMNTKYDENDKLIREVKVITLKSKLVSDFRKDFQFYKVREINNYHHAHDAYLNAVVGTALIKKYPKLESEFVYGDYKVYDVRKMIAKSEQEIGKATAKYFFYSNIMNFFKTEITLANGEIRKRPLIETNGETGEIVWDKGRDFATVRKVLSMPQVNIVKKTEVQTGGFSKESILPKRNSDKLIARKKDWDPKKYGGFDSPTVAYSVLVVAKVEKGKSKKLKSVKELLGITIMERSSFEKNPIDFLEAKGYKEVKKDLIIKLPKYSLFELENGRKRMLASAGELQKGNELALPSKYVNFLYLASHYEKLKGSPEDNEQKQLFVEQHKHYLDEIIEQISEFSKRVILADANLDKVLSAYNKHRDKPIREQAENIIHLFTLTNLGAPAAFKYFDTTIDRKRYTSTKEVLDATLIHQSITGLYETRIDLSQLGGDKRPAATKKAGQAKKKK

SEQ ID NO: 36 - DNA, 4176 bp, Artificial Sequence
  Synthetic
  misc_feature (1)..(3): Start Codon
  misc_feature (10)..(30): 5' NLS
  misc_feature (4126)..(4173): 3' NLS
  misc_feature (4174)..(4176): Stop Codon
atggacaagcccaagaaaaagcggaaagtgaagtacagcatcggcctggacatcggcaccaactctgtgggctgggccgtgatcaccgacgagtacaaggtgcccagcaagaaattcaaggtgctgggcaacaccgacaggcacagcatcaagaagaacctgatcggcgccctgctgttcgacagcggcgaaacagccgaggccaccagactgaagagaaccgccagaagaagatacaccaggcggaagaacaggatctgctatctgcaagagatcttcagcaacgagatggccaaggtggacgacagcttcttccacagactggaagagtccttcctggtggaagaggacaagaagcacgagagacaccccatcttcggcaacatcgtggacgaggtggcctaccacgagaagtaccccaccatctaccacctgagaaagaaactggtggacagcaccgacaaggccgacctgagactgatctacctggccctggcccacatgatcaagttcagaggccacttcctgatcgagggcgacctgaaccccgacaacagcgacgtggacaagctgttcatccagctggtgcagacctacaaccagctgttcgaggaaaaccccatcaacgccagcggcgtggacgccaaggctatcctgtctgccagactgagcaagagcagaaggctggaaaatctgatcgcccagctgcccggcgagaagaagaacggcctgttcggcaacctgattgccctgagcctgggcctgacccccaacttcaagagcaacttcgacctggccgaggatgccaaactgcagctgagcaaggacacctacgacgacgacctggacaacctgctggcccagatcggcgaccagtacgccgacctgttcctggccgccaagaacctgtctgacgccatcctgctgagcgacatcctgagagtgaacaccgagatcaccaaggcccccctgagcgcctctatgatcaagagatacgacgagcaccaccaggacctgaccctgctgaaagctctcgtgcggcagcagctgcctgagaagtacaaagaaatcttcttcgaccagagcaagaacggctacgccggctacatcgatggcggcgctagccaggaagagttctacaagttcatcaagcccatcctggaaaagatggacggcaccgaggaactgctcgtgaagctgaacagagaggacctgctgagaaagcagagaaccttcgacaacggcagcatcccccaccagatccacctgggagagctgcacgctatcctgagaaggcaggaagatttttacccattcctgaaggacaaccgggaaaagatcgagaagatcctgaccttcaggatcccctactacgtgggccccctggccagaggcaacagcagattcgcctggatgaccagaaagagcgaggaaaccatcaccccctggaacttcgaggaagtggtggacaagggcgccagcgcccagagcttcatcgagagaatgacaaacttcgataagaacctgcccaacgagaaggtgctgcccaagcacagcctgctgtacgagtacttcaccgtgtacaacgagctgaccaaagtgaaatacgtgaccgagggaatgagaaagcccgccttcctgagcggcgagcagaaaaaggccatcgtggacctgctgttcaagaccaacagaaaagtgaccgtgaagcagctgaaagaggactacttcaagaaaatcgagtgcttcgactccgtggaaatctccggcgtggaagatagattcaacgcctccctgggcacataccacgatctgctgaaaattatcaaggacaaggacttcctggataacgaagagaacgaggacattctggaagatatcgtgctgaccctgacactgtttgaggaccgcgagatgatcgaggaaaggctgaaaacctacgctcacctgttcgacgacaaagtgatgaagcagctgaagagaaggcggtacaccggctggggcaggctgagcagaaagctgatcaacggcatcagagacaagcagagcggcaagacaatcctggatttcctgaagtccgacggcttcgccaaccggaacttcatgcagctgatccacgacgacagcctgacattcaaagaggacatccagaaagcccaggtgtccggccagggcgactctctgcacgagcatatcgctaacctggccggcagccccgctatcaagaagggcatcctgcagacagtgaaggtggtggacgagctcgtgaaagtgatgggcagacacaagcccgagaacatcgtgatcgagatggctagagagaaccagaccacccagaagggacagaagaactcccgcgagaggatgaagagaatcgaagagggcatcaaagagctgggcagccagatcctgaaagaacaccccgtggaaaacacccagctgcagaacgagaagctgtacctgtactacctgcagaatggccgggatatgtacgtggaccaggaactggacatcaacagactgtccgactacgatgtggaccatatcgtgcctcagagctttctgaaggacgactccatcgataacaaagtgctgactcggagcgacaagaacagaggcaagagcgacaacgtgccctccgaagaggtcgtgaagaagatgaagaactactggcgacagctgctgaacgccaagctgattacccagaggaagttcgataacctgaccaaggccgagagaggcggcctgagcgagctggataaggccggcttcatcaagaggcagctggtggaaaccagacagatcacaaagcacgtggcacagatcctggactcccggatgaacactaagtacgacgaaaacgataagctgatccgggaagtgaaagtgatcaccctgaagtccaagctggtgtccgatttccggaaggatttccagttttacaaagtgcgcgagatcaacaactaccaccacgcccacgacgcctacctgaacgccgtcgtgggaaccgccctgatcaaaaagtaccctaagctggaaagcgagttcgtgtacggcgactacaaggtgtacgacgtgcggaagatgatcgccaagagcgagcaggaaatcggcaaggctaccgccaagtacttcttctacagcaacatcatgaactttttcaagaccgaaatcaccctggccaacggcgagatcagaaagcgccctctgatcgagacaaacggcgaaaccggggagatcgtgtgggataagggcagagacttcgccacagtgcgaaaggtgctgagcatgccccaagtgaatatcgtgaaaaagaccgaggtgcagacaggcggcttcagcaaagagtctatcctgcccaagaggaacagcgacaagctgatcgccagaaagaaggactgggaccccaagaagtacggcggcttcgacagccctaccgtggcctactctgtgctggtggtggctaaggtggaaaagggcaagtccaagaaactgaagagtgtgaaagagctgctggggatcaccatcatggaaagaagcagctttgagaagaaccctatcgactttctggaagccaagggctacaaagaagtgaaaaaggacctgatcatcaagctgcctaagtactccctgttcgagctggaaaacggcagaaagagaatgctggcctctgccggcgaactgcagaagggaaacgagctggccctgcctagcaaatatgtgaacttcctgtacctggcctcccactatgagaagctgaagggcagccctgaggacaacgaacagaaacagctgtttgtggaacagcataagcactacctggacgagatcatcgagcagatcagcgagttctccaagagagtgatcctggccgacgccaatctggacaaggtgctgtctgcctacaacaagcacagggacaagcctatcagagagcaggccgagaatatcatccacctgttcaccctgacaaacctgggcgctcctgccgccttcaagtactttgacaccaccatcgaccggaagaggtacaccagcaccaaagaggtgctggacgccaccctgatccaccagagcatcaccggcctgtacgagacaagaatcgacctgtctcagctgggaggcgacaagagacctgccgccactaagaaggccggacaggccaaaaagaagaagtga

SEQ ID NO: 37 - RNA, 16 nt, Artificial Sequence
  Synthetic
guuuuagagcuaugcu

SEQ ID NO: 38 - RNA, 67 nt, Artificial Sequence
  Synthetic
agcauagcaaguuaaaauaaggcuaguccguuaucaacuugaaaaaguggcaccgagucggugcuuu

SEQ ID NO: 39 - RNA, 77 nt, Artificial Sequence
  Synthetic
guuuuagagcuagaaauagcaaguuaaaauaaggcuaguccguuaucaacuugaaaaaguggcaccgagucggugcu

SEQ ID NO: 40 - RNA, 82 nt, Artificial Sequence
  Synthetic
guuggaaccauucaaaacagcauagcaaguuaaaauaaggcuaguccguuaucaacuugaaaaaguggcaccgagucggugc

SEQ ID NO: 41 - RNA, 76 nt, Artificial Sequence
  Synthetic
guuuuagagcuagaaauagcaaguuaaaauaaggcuaguccguuaucaacuugaaaaaguggcaccgagucggugc

SEQ ID NO: 42 - RNA, 86 nt, Artificial Sequence
  Synthetic
guuuaagagcuaugcuggaaacagcauagcaaguuuaaauaaggcuaguccguuaucaacuugaaaaaguggcaccgagucggugc

SEQ ID NO: 43 - DNA, 23 bp, Artificial Sequence
  Synthetic
  misc_feature (2)..(21): n is a, c, g, or t
gnnnnnnnnnnnnnnnnnnnngg

SEQ ID NO: 44 - DNA, 23 bp, Artificial Sequence
  Synthetic
  misc_feature (1)..(21): n is a, c, g, or t
nnnnnnnnnnnnnnnnnnnnngg

SEQ ID NO: 45 - DNA, 25 bp, Artificial Sequence
  Synthetic
  misc_feature (3)..(23): n is a, c, g, or t
ggnnnnnnnnnnnnnnnnnnnnngg

SEQ ID NO: 46 - protein, 615 aa, Homo sapiens
  MISC_FEATURE (1)..(19): Signal Peptide
  MISC_FEATURE (20)..(372): Heavy Chain
  MISC_FEATURE (373)..(615): Light Chain
MRALLLLGFLLVSLESTLSIPPWEAPKEHKYKAEEHTVVLTVTGEPCHFPFQYHRQLYHKCTHKGRPGPQPWCATTPNFDQDQRWGYCLEPKKVKDHCSKHSPCQKGGTCVNMPSGPHCLCPQHLTGNHCQKEKCFEPQLLRFFHKNEIWYRTEQAAVARCQCKGPDAHCQRLASQACRTNPCLHGGRCLEVEGHRLCHCPVGYTGAFCDVDTKASCYDGRGLSYRGLARTTLSGAPCQPWASEATYRNVTAEQARNWGLGGHAFCRNPDNDIRPWCFVLNRDRLSWEYCDLAQCQTPTQAAPPTPVSPRLHVPLMPAQPAPPKPQPTTRTPPQSQTPGALPAKREQPPSLTRNGPLSCGQRLRKSLSSMTRVVGGLVALRGAHPYIAALYWGHSFCAGSLIAPCWVLTAAHCLQDRPAPEDLTVVLGQERRNHSCEPCQTLAVRSYRLHEAFSPVSYQHDLALLRLQEDADGSCALLSPYVQPVCLPSGAARPSETTLCQVAGWGHQFEGAEEYASFLQEAQVPFLSLERCSAPDVHGSSILPGMLCAGFLEGGTDACQGDSGGPLVCEDQAAERRLTLQGIISWGSGCGDRNKPGVYTDVAYYLAWIREHTVS

SEQ ID NO: 47 - protein, 353 aa, Homo sapiens
IPPWEAPKEHKYKAEEHTVVLTVTGEPCHFPFQYHRQLYHKCTHKGRPGPQPWCATTPNFDQDQRWGYCLEPKKVKDHCSKHSPCQKGGTCVNMPSGPHCLCPQHLTGNHCQKEKCFEPQLLRFFHKNEIWYRTEQAAVARCQCKGPDAHCQRLASQACRTNPCLHGGRCLEVEGHRLCHCPVGYTGAFCDVDTKASCYDGRGLSYRGLARTTLSGAPCQPWASEATYRNVTAEQARNWGLGGHAFCRNPDNDIRPWCFVLNRDRLSWEYCDLAQCQTPTQAAPPTPVSPRLHVPLMPAQPAPPKPQPTTRTPPQSQTPGALPAKREQPPSLTRNGPLSCGQRLRKSLSSMTR

SEQ ID NO: 48 - DNA, 1848 bp, Homo sapiens
  misc_feature (1)..(57): Signal Peptide
  misc_feature (58)..(1116): Heavy Chain
  misc_feature (1117)..(1845): Light Chain
atgagggctctgctgctcctggggttcctgctggtgagcttggagtcaacactttcgattccaccttgggaagcccccaaggagcataagtacaaagctgaagagcacacagtcgttctcactgtcaccggggagccctgccacttccccttccagtaccaccggcagctgtaccacaaatgtacccacaagggccggccaggccctcagccctggtgtgctaccacccccaactttgatcaggaccagcgatggggatactgtttggagcccaagaaagtgaaagaccactgcagcaaacacagcccctgccagaaaggagggacctgtgtgaacatgccaagcggcccccactgtctctgtccacaacacctcactggaaaccactgccagaaagagaagtgctttgagcctcagcttctccggtttttccacaagaatgagatatggtatagaactgagcaagcagctgtggccagatgccagtgcaagggtcctgatgcccactgccagcggctggccagccaggcctgccgcaccaacccgtgcctccatgggggtcgctgcctagaggtggagggccaccgcctgtgccactgcccggtgggctacaccggagccttctgcgacgtggacaccaaggcaagctgctatgatggccgcgggctcagctaccgcggcctggccaggaccacgctctcgggtgcgccctgtcagccgtgggcctcggaggccacctaccggaacgtgactgccgagcaagcgcggaactggggactgggcggccacgccttctgccggaacccggacaacgacatccgcccgtggtgcttcgtgctgaaccgcgaccggctgagctgggagtactgcgacctggcacagtgccagaccccaacccaggcggcgcctccgaccccggtgtcccctaggcttcatgtcccactcatgcccgcgcagccggcaccgccgaagcctcagcccacgacccggaccccgcctcagtcccagaccccgggagccttgccggcgaagcgggagcagccgccttccctgaccaggaacggcccactgagctgcgggcagcggctccgcaagagtctgtcttcgatgacccgcgtcgttggcgggctggtggcgctacgcggggcgcacccctacatcgccgcgctgtactggggccacagtttctgcgccggcagcctcatcgccccctgctgggtgctgacggccgctcactgcctgcaggaccggcccgcacccgaggatctgacggtggtgctcggccaggaacgccgtaaccacagctgtgagccgtgccagacgttggccgtgcgctcctaccgcttgcacgaggccttctcgcccgtcagctaccagcacgacctggctctgttgcgccttcaggaggatgcggacggcagctgcgcgctcctgtcgccttacgttcagccggtgtgcctgccaagcggcgccgcgcgaccctccgagaccacgctctgccaggtggccggctggggccaccagttcgagggggcggaggaatatgccagcttcctgcaggaggcgcaggtaccgttcctctccctggagcgctgctcagccccggacgtgcacggatcctccatcctccccggcatgctctgcgcagggttcctcgagggcggcaccgatgcgtgccagggtgattccggaggcccgctggtgtgtgaggaccaagctgcagagcgccggctcaccctgcaaggcatcatcagctggggatcgggctgtggtgaccgcaacaagccaggcgtctacaccgatgtggcctactacctggcctggatccgggagcacaccgtttcctga

SEQ ID NO: 49 - DNA, 1059 bp, Homo sapiens
attccaccttgggaagcccccaaggagcataagtacaaagctgaagagcacacagtcgttctcactgtcaccggggagccctgccacttccccttccagtaccaccggcagctgtaccacaaatgtacccacaagggccggccaggccctcagccctggtgtgctaccacccccaactttgatcaggaccagcgatggggatactgtttggagcccaagaaagtgaaagaccactgcagcaaacacagcccctgccagaaaggagggacctgtgtgaacatgccaagcggcccccactgtctctgtccacaacacctcactggaaaccactgccagaaagagaagtgctttgagcctcagcttctccggtttttccacaagaatgagatatggtatagaactgagcaagcagctgtggccagatgccagtgcaagggtcctgatgcccactgccagcggctggccagccaggcctgccgcaccaacccgtgcctccatgggggtcgctgcctagaggtggagggccaccgcctgtgccactgcccggtgggctacaccggagccttctgcgacgtggacaccaaggcaagctgctatgatggccgcgggctcagctaccgcggcctggccaggaccacgctctcgggtgcgccctgtcagccgtgggcctcggaggccacctaccggaacgtgactgccgagcaagcgcggaactggggactgggcggccacgccttctgccggaacccggacaacgacatccgcccgtggtgcttcgtgctgaaccgcgaccggctgagctgggagtactgcgacctggcacagtgccagaccccaacccaggcggcgcctccgaccccggtgtcccctaggcttcatgtcccactcatgcccgcgcagccggcaccgccgaagcctcagcccacgacccggaccccgcctcagtcccagaccccgggagccttgccggcgaagcgggagcagccgccttccctgaccaggaacggcccactgagctgcgggcagcggctccgcaagagtctgtcttcgatgacccgc

SEQ ID NO: 50 - DNA, 18 bp, Artificial Sequence
  Synthetic
tggaccaacggacggatg

SEQ ID NO: 51 - DNA, 18 bp, Artificial Sequence
  Synthetic
tgccacttccccttccag

SEQ ID NO: 52 - DNA, 21 bp, Artificial Sequence
  Synthetic
actgtctctgtccacaacacc

SEQ ID NO: 53 - DNA, 18 bp, Artificial Sequence
  Synthetic
accaacccgtgcctccat

SEQ ID NO: 54 - DNA, 19 bp, Artificial Sequence
  Synthetic
gtggtgcttcgtgctgaac

SEQ ID NO: 55 - DNA, 20 bp, Artificial Sequence
  Synthetic
aggatctgacggtggtgctc

SEQ ID NO: 56 - DNA, 20 bp, Artificial Sequence
  Synthetic
acaccgatgtggcctactac

SEQ ID NO: 57 - DNA, 20 bp, Artificial Sequence
  Synthetic
ccaggtggtctcctctgact

SEQ ID NO: 58 - DNA, 21 bp, Artificial Sequence
  Synthetic
cccaaggtggaatcgaaagtg

SEQ ID NO: 59 - DNA, 19 bp, Artificial Sequence
  Synthetic
gtagcacaccagggctgag

SEQ ID NO: 60 - DNA, 21 bp, Artificial Sequence
  Synthetic
cggagaagctgaggctcaaag

SEQ ID NO: 61 - DNA, 19 bp, Artificial Sequence
  Synthetic
gcagaaggctccggtgtag

SEQ ID NO: 62 - DNA, 19 bp, Artificial Sequence
  Synthetic
gttggggtctggcactgtg

SEQ ID NO: 63 - DNA, 19 bp, Artificial Sequence
  Synthetic
gtagctgacgggcgagaag

SEQ ID NO: 64 - DNA, 19 bp, Artificial Sequence
  Synthetic
actgcggaatcaccaagga

SEQ ID NO: 65 - DNA, 21 bp, Artificial Sequence
  Synthetic
gcttgacaaagtggtcgttga

SEQ ID NO: 66 - DNA, 23 bp, Artificial Sequence
  Synthetic
catgagggctctgctgctcctgg

SEQ ID NO: 67 - DNA, 24 bp, Artificial Sequence
  Synthetic
accaccggcagctgtaccacaaat

SEQ ID NO: 68 - DNA, 27 bp, Artificial Sequence
  Synthetic
tcactggaaaccactgccagaaagaga

SEQ ID NO: 69 - DNA, 23 bp, Artificial Sequence
  Synthetic
ctgcctagaggtggagggccacc

SEQ ID NO: 70 - DNA, 23 bp, Artificial Sequence
  Synthetic
cgaccggctgagctgggagtact

SEQ ID NO: 71 - DNA, 23 bp, Artificial Sequence
  Synthetic
ccaggaacgccgtaaccacagct

SEQ ID NO: 72 - DNA, 23 bp, Artificial Sequence
  Synthetic
ctggatccgggagcacaccgttt

SEQ ID NO: 73 - DNA, 22 bp, Artificial Sequence
  Synthetic
tcaacagcgacacccactcctc

SEQ ID NO: 74 - protein, 300 aa, Homo sapiens
MPAQPAPPKPQPTTRTPPQSQTPGALPAKREQPPSLTRNGPLSCGQRLRKSLSSMTRVVGGLVALRGAHPYIAALYWGHSFCAGSLIAPCWVLTAAHCLQDRPAPEDLTVVLGQERRNHSCEPCQTLAVRSYRLHEAFSPVSYQHDLALLRLQEDADGSCALLSPYVQPVCLPSGAARPSETTLCQVAGWGHQFEGAEEYASFLQEAQVPFLSLERCSAPDVHGSSILPGMLCAGFLEGGTDACQGDSGGPLVCEDQAAERRLTLQGIISWGSGCGDRNKPGVYTDVAYYLAWIREHTVS

SEQ ID NO: 75 - DNA, 903 bp, Homo sapiens
atgcccgcgcagccggcaccgccgaagcctcagcccacgacccggaccccgcctcagtcccagaccccgggagccttgccggcgaagcgggagcagccgccttccctgaccaggaacggcccactgagctgcgggcagcggctccgcaagagtctgtcttcgatgacccgcgtcgttggcgggctggtggcgctacgcggggcgcacccctacatcgccgcgctgtactggggccacagtttctgcgccggcagcctcatcgccccctgctgggtgctgacggccgctcactgcctgcaggaccggcccgcacccgaggatctgacggtggtgctcggccaggaacgccgtaaccacagctgtgagccgtgccagacgttggccgtgcgctcctaccgcttgcacgaggccttctcgcccgtcagctaccagcacgacctggctctgttgcgccttcaggaggatgcggacggcagctgcgcgctcctgtcgccttacgttcagccggtgtgcctgccaagcggcgccgcgcgaccctccgagaccacgctctgccaggtggccggctggggccaccagttcgagggggcggaggaatatgccagcttcctgcaggaggcgcaggtaccgttcctctccctggagcgctgctcagccccggacgtgcacggatcctccatcctccccggcatgctctgcgcagggttcctcgagggcggcaccgatgcgtgccagggtgattccggaggcccgctggtgtgtgaggaccaagctgcagagcgccggctcaccctgcaaggcatcatcagctggggatcgggctgtggtgaccgcaacaagccaggcgtctacaccgatgtggcctactacctggcctggatccgggagcacaccgtttcctga

SEQ ID NO: 76 - protein, 246 aa, Homo sapiens [sequence omitted]

SEQ ID NO: 77 - DNA, 741 bp, Homo sapiens
atgacccgcgtcgttggcgggctggtggcgctacgcggggcgcacccctacatcgccgcgctgtactggggccacagtttctgcgccggcagcctcatcgccccctgctgggtgctgacggccgctcactgcctgcaggaccggcccgcacccgaggatctgacggtggtgctcggccaggaacgccgtaaccacagctgtgagccgtgccagacgttggccgtgcgctcctaccgcttgcacgaggccttctcgcccgtcagctaccagcacgacctggctctgttgcgccttcaggaggatgcggacggcagctgcgcgctcctgtcgccttacgttcagccggtgtgcctgccaagcggcgccgcgcgaccctccgagaccacgctctgccaggtggccggctggggccaccagttcgagggggcggaggaatatgccagcttcctgcaggaggcgcaggtaccgttcctctccctggagcgctgctcagccccggacgtgcacggatcctccatcctccccggcatgctctgcgcagggttcctcgagggcggcaccgatgcgtgccagggtgattccggaggcccgctggtgtgtgaggaccaagctgcagagcgccggctcaccctgcaaggcatcatcagctggggatcgggctgtggtgaccgcaacaagccaggcgtctacaccgatgtggcctactacctggcctggatccgggagcacaccgtttcctga

SEQ ID NO: 78 - protein, 70 aa, Homo sapiens
MLCAGFLEGGTDACQGDSGGPLVCEDQAAERRLTLQGIISWGSGCGDRNKPGVYTDVAYYLAWIREHTVS

SEQ ID NO: 79 - DNA, 213 bp, Homo sapiens
atgctctgcgcagggttcctcgagggcggcaccgatgcgtgccagggtgattccggaggcccgctggtgtgtgaggaccaagctgcagagcgccggctcaccctgcaaggcatcatcagctggggatcgggctgtggtgaccgcaacaagccaggcgtctacaccgatgtggcctactacctggcctggatccgggagcacaccgtttcctga

SEQ ID NO: 80 - RNA, 72 nt, Artificial Sequence
  Synthetic
aaacagcauagcaaguuaaaauaaggcuaguccguuaucaacuugaaaaaguggcaccgagucggugcuuuu

SEQ ID NO: 81 - RNA, 82 nt, Artificial Sequence; identical to SEQ ID NO: 40
  Synthetic

SEQ ID NO: 82 - RNA, 83 nt, Artificial Sequence
  Synthetic
guuuuagagcuagaaauagcaaguuaaaauaaggcuaguccguuaucaacuugaaaaaguggcaccgagucggugcuuuuuuu

SEQ ID NO: 83 - RNA, 80 nt, Artificial Sequence
  Synthetic
guuuuagagcuagaaauagcaaguuaaaauaaggcuaguccguuaucaacuugaaaaaguggcaccgagucggugcuuuu

SEQ ID NO: 84 - RNA, 92 nt, Artificial Sequence
  Synthetic
guuuaagagcuaugcuggaaacagcauagcaaguuuaaauaaggcuaguccguuaucaacuugaaaaaguggcaccgagucggugcuuuuuu